European Patent Application EP 4 644 552 A1, published November 5, 2025. Title: POLYNUCLEOTIDE MOLECULE FOR PREVENTING OR TREATING HPV INFECTION-RELATED DISEASES. Applicant: RINUAGENE BIOTECHNOLOGY CO., LTD. The sequence listing filed with the application follows.

SEQUENCE LISTING (54 sequences)

SEQ ID NO: 1 - protein, 85 aa, synthetic construct
MHQKRTAMFQDPQERPRKLPHLCTELQTTIHDIILECVYCKQQLLRREVYDFAFRDLCIVYRDGNPYAVCDKCLKFYSKISEYRY

SEQ ID NO: 2 - protein, 65 aa, synthetic construct
MHGDTPTLHEYMLDLQPETTDLYCYEQLNDSSEEEDEIDGPAGQAEPDRAHYNIVTFCCKCDSTL

SEQ ID NO: 3 - protein, 88 aa, synthetic construct
DKCLKFYSKISEYRYYCYSVYGTTLEQQYNKPLCDLLIRCINCQKPLCPEEKQRHLDKKQRFHNIRGRWTGRCMSCCRSSRTRRETQL

SEQ ID NO: 4 - protein, 48 aa, synthetic construct
HYNIVTFCCKCDSTLRLCVQSTHVDIRTLEDLLMGTLGIVCPICSQKP

SEQ ID NO: 5 - protein, 85 aa, synthetic construct
MARFEDPTRRPYKLPDLCTELNTSLQDIEITCVYCKTVLELTEVFEFAFKDLFVVYRDSIPHAACHKCIDFYSRIRELRYYSDSV

SEQ ID NO: 6 - protein, 65 aa, synthetic construct
MYGPKATLQDIVLHLEPQNEIPVDLLCHEQLSDSEEENDEIDGVNHQHLPARRAEPQRHTMLCMC

SEQ ID NO: 7 - protein, 88 aa, synthetic construct
FYSRIRELRYYSDSVYGDTLEKLTNTGLYNLLIRCLRCQKPLNPAEKLRHLNEKRRFHKIAGHYRGQCHSCCNRARQERLQRRRETQV

SEQ ID NO: 8 - protein, 55 aa, synthetic construct
ARRAEPQRHTMLCMCCKCEARIELVVESSADDLRAFQQLFLSTLSFVCPWCASQQ

SEQ ID NO: 9 - protein, 306 aa, synthetic construct
MNVCQDKILEHYENDSKDILEHYENDSKDLCDHICDHIDYWKHIRLECAIMYKARIRLECAIMYKAREMGFHQFDGDICNTMHYTNWIYICEDAQCTVVEGQVDKKWEVHAGGQVILCPESGQRRIKRPRSENCHPNKLLILKCLRYRFKKHCKLSSTWHWTCHDGKHKWHWTCHDGKHKNAIVTLTYDHIDYWKAIRQENAIFFAARHQVVPALNICKAKACKAIEWNTEPKHCFKKGGQHIEVWFDYVAWDSVYYCGDDGWCKTEAEKYGCKGTWEVHFGNSIDCNDSMCSTFDDNVSATELVK

SEQ ID NO: 10 - protein, 163 aa, synthetic construct
ITQDCSFQHSPISSDFAVKIRELSDYLLQDYPVTVASNLQDEELCGGLWRLVLAQRWMERLKTVAGSKMQGLLERVNTEIHFVTKCAFQPPPSCLRFVQTNISRLLQETSEQLVALKPWITRQNFSRCLELQCQPDSSTLPPPWSPRPLEATAPTAPGGGSGD

SEQ ID NO: 11 - protein, 23 aa, synthetic construct
MDAMKRGLCCVLLLCGAVFVSPS

SEQ ID NO: 12 - protein, 579 aa, synthetic construct
MHQKRTAMFQDPQERPRKLPHLCTELQTTIHDIILECVYCKQQLLRREVYDFAFRDLCIVYRDGNPYAVCDKCLKFYSKISEYRYMHGDTPTLHEYMLDLQPETTDLYCYEQLNDSSEEEDEIDGPAGQAEPDRAHYNIVTFCCKCDSTLDKCLKFYSKISEYRYYCYSVYGTTLEQQYNKPLCDLLIRCINCQKPLCPEEKQRHLDKKQRFHNIRGRWTGRCMSCCRSSRTRRETQLHYNIVTFCCKCDSTLRLCVQSTHVDIRTLEDLLMGTLGIVCPICSQKPMARFEDPTRRPYKLPDLCTELNTSLQDIEITCVYCKTVLELTEVFEFAFKDLFVVYRDSIPHAACHKCIDFYSRIRELRYYSDSVMYGPKATLQDIVLHLEPQNEIPVDLLCHEQLSDSEEENDEIDGVNHQHLPARRAEPQRHTMLCMCFYSRIRELRYYSDSVYGDTLEKLTNTGLYNLLIRCLRCQKPLNPAEKLRHLNEKRRFHKIAGHYRGQCHSCCNRARQERLQRRRETQVARRAEPQRHTMLCMCCKCEARIELVVESSADDLRAFQQLFLSTLSFVCPWCASQQ

SEQ ID NO: 13 - protein, 579 aa, synthetic construct
MARFEDPTRRPYKLPDLCTELNTSLQDIEITCVYCKTVLELTEVFEFAFKDLFVVYRDSIPHAACHKCIDFYSRIRELRYYSDSVMYGPKATLQDIVLHLEPQNEIPVDLLCHEQLSDSEEENDEIDGVNHQHLPARRAEPQRHTMLCMCFYSRIRELRYYSDSVYGDTLEKLTNTGLYNLLIRCLRCQKPLNPAEKLRHLNEKRRFHKIAGHYRGQCHSCCNRARQERLQRRRETQVARRAEPQRHTMLCMCCKCEARIELVVESSADDLRAFQQLFLSTLSFVCPWCASQQMHQKRTAMFQDPQERPRKLPHLCTELQTTIHDIILECVYCKQQLLRREVYDFAFRDLCIVYRDGNPYAVCDKCLKFYSKISEYRYMHGDTPTLHEYMLDLQPETTDLYCYEQLNDSSEEEDEIDGPAGQAEPDRAHYNIVTFCCKCDSTLDKCLKFYSKISEYRYYCYSVYGTTLEQQYNKPLCDLLIRCINCQKPLCPEEKQRHLDKKQRFHNIRGRWTGRCMSCCRSSRTRRETQLHYNIVTFCCKCDSTLRLCVQSTHVDIRTLEDLLMGTLGIVCPICSQKP

SEQ ID NO: 14 - protein, 591 aa, synthetic construct
MHQKRTAMFQDPQERPRKLPHLCTELQTTIHDIILECVYCKQQLLRREVYDFAFRDLCIVYRDGNPYAVCDKCLKFYSKISEYRYAAMHGDTPTLHEYMLDLQPETTDLYCYEQLNDSSEEEDEIDGPAGQAEPDRAHYNIVTFCCKCDSTLAADKCLKFYSKISEYRYYCYSVYGTTLEQQYNKPLCDLLIRCINCQKPLCPEEKQRHLDKKQRFHNIRGRWTGRCMSCCRSSRTRRETQLAAHYNIVTFCCKCDSTLRLCVQSTHVDIRTLEDLLMGTLGIVCPICSQKPMARFEDPTRRPYKLPDLCTELNTSLQDIEITCVYCKTVLELTEVFEFAFKDLFVVYRDSIPHAACHKCIDFYSRIRELRYYSDSVAAMYGPKATLQDIVLHLEPQNEIPVDLLCHEQLSDSEEENDEIDGVNHQHLPARRAEPQRHTMLCMCAAFYSRIRELRYYSDSVYGDTLEKLTNTGLYNLLIRCLRCQKPLNPAEKLRHLNEKRRFHKIAGHYRGQCHSCCNRARQERLQRRRETQVAAARRAEPQRHTMLCMCCKCEARIELVVESSADDLRAFQQLFLSTLSFVCPWCASQQ

SEQ ID NO: 15 - protein, 885 aa, synthetic construct
MNVCQDKILEHYENDSKDILEHYENDSKDLCDHICDHIDYWKHIRLECAIMYKARIRLECAIMYKAREMGFHQFDGDICNTMHYTNWIYICEDAQCTVVEGQVDKKWEVHAGGQVILCPESGQRRIKRPRSENCHPNKLLILKCLRYRFKKHCKLSSTWHWTCHDGKHKWHWTCHDGKHKNAIVTLTYDHIDYWKAIRQENAIFFAARHQVVPALNICKAKACKAIEWNTEPKHCFKKGGQHIEVWFDYVAWDSVYYCGDDGWCKTEAEKYGCKGTWEVHFGNSIDCNDSMCSTFDDNVSATELVKMHQKRTAMFQDPQERPRKLPHLCTELQTTIHDIILECVYCKQQLLRREVYDFAFRDLCIVYRDGNPYAVCDKCLKFYSKISEYRYMHGDTPTLHEYMLDLQPETTDLYCYEQLNDSSEEEDEIDGPAGQAEPDRAHYNIVTFCCKCDSTLDKCLKFYSKISEYRYYCYSVYGTTLEQQYNKPLCDLLIRCINCQKPLCPEEKQRHLDKKQRFHNIRGRWTGRCMSCCRSSRTRRETQLHYNIVTFCCKCDSTLRLCVQSTHVDIRTLEDLLMGTLGIVCPICSQKPMARFEDPTRRPYKLPDLCTELNTSLQDIEITCVYCKTVLELTEVFEFAFKDLFVVYRDSIPHAACHKCIDFYSRIRELRYYSDSVMYGPKATLQDIVLHLEPQNEIPVDLLCHEQLSDSEEENDEIDGVNHQHLPARRAEPQRHTMLCMCFYSRIRELRYYSDSVYGDTLEKLTNTGLYNLLIRCLRCQKPLNPAEKLRHLNEKRRFHKIAGHYRGQCHSCCNRARQERLQRRRETQVARRAEPQRHTMLCMCCKCEARIELVVESSADDLRAFQQLFLSTLSFVCPWCASQQ

SEQ ID NO: 16 - protein, 885 aa, synthetic construct
MNVCQDKILEHYENDSKDILEHYENDSKDLCDHICDHIDYWKHIRLECAIMYKARIRLECAIMYKAREMGFHQFDGDICNTMHYTNWIYICEDAQCTVVEGQVDKKWEVHAGGQVILCPESGQRRIKRPRSENCHPNKLLILKCLRYRFKKHCKLSSTWHWTCHDGKHKWHWTCHDGKHKNAIVTLTYDHIDYWKAIRQENAIFFAARHQVVPALNICKAKACKAIEWNTEPKHCFKKGGQHIEVWFDYVAWDSVYYCGDDGWCKTEAEKYGCKGTWEVHFGNSIDCNDSMCSTFDDNVSATELVKMARFEDPTRRPYKLPDLCTELNTSLQDIEITCVYCKTVLELTEVFEFAFKDLFVVYRDSIPHAACHKCIDFYSRIRELRYYSDSVMYGPKATLQDIVLHLEPQNEIPVDLLCHEQLSDSEEENDEIDGVNHQHLPARRAEPQRHTMLCMCFYSRIRELRYYSDSVYGDTLEKLTNTGLYNLLIRCLRCQKPLNPAEKLRHLNEKRRFHKIAGHYRGQCHSCCNRARQERLQRRRETQVARRAEPQRHTMLCMCCKCEARIELVVESSADDLRAFQQLFLSTLSFVCPWCASQQMHQKRTAMFQDPQERPRKLPHLCTELQTTIHDIILECVYCKQQLLRREVYDFAFRDLCIVYRDGNPYAVCDKCLKFYSKISEYRYMHGDTPTLHEYMLDLQPETTDLYCYEQLNDSSEEEDEIDGPAGQAEPDRAHYNIVTFCCKCDSTLDKCLKFYSKISEYRYYCYSVYGTTLEQQYNKPLCDLLIRCINCQKPLCPEEKQRHLDKKQRFHNIRGRWTGRCMSCCRSSRTRRETQLHYNIVTFCCKCDSTLRLCVQSTHVDIRTLEDLLMGTLGIVCPICSQKP

SEQ ID NO: 17 - protein, 765 aa, synthetic construct
MDAMKRGLCCVLLLCGAVFVSPSITQDCSFQHSPISSDFAVKIRELSDYLLQDYPVTVASNLQDEELCGGLWRLVLAQRWMERLKTVAGSKMQGLLERVNTEIHFVTKCAFQPPPSCLRFVQTNISRLLQETSEQLVALKPWITRQNFSRCLELQCQPDSSTLPPPWSPRPLEATAPTAPGGGSGDMHQKRTAMFQDPQERPRKLPHLCTELQTTIHDIILECVYCKQQLLRREVYDFAFRDLCIVYRDGNPYAVCDKCLKFYSKISEYRYMHGDTPTLHEYMLDLQPETTDLYCYEQLNDSSEEEDEIDGPAGQAEPDRAHYNIVTFCCKCDSTLDKCLKFYSKISEYRYYCYSVYGTTLEQQYNKPLCDLLIRCINCQKPLCPEEKQRHLDKKQRFHNIRGRWTGRCMSCCRSSRTRRETQLHYNIVTFCCKCDSTLRLCVQSTHVDIRTLEDLLMGTLGIVCPICSQKPMARFEDPTRRPYKLPDLCTELNTSLQDIEITCVYCKTVLELTEVFEFAFKDLFVVYRDSIPHAACHKCIDFYSRIRELRYYSDSVMYGPKATLQDIVLHLEPQNEIPVDLLCHEQLSDSEEENDEIDGVNHQHLPARRAEPQRHTMLCMCFYSRIRELRYYSDSVYGDTLEKLTNTGLYNLLIRCLRCQKPLNPAEKLRHLNEKRRFHKIAGHYRGQCHSCCNRARQERLQRRRETQVARRAEPQRHTMLCMCCKCEARIELVVESSADDLRAFQQLFLSTLSFVCPWCASQQ

SEQ ID NO: 18 - protein, 765 aa, synthetic construct
MDAMKRGLCCVLLLCGAVFVSPSITQDCSFQHSPISSDFAVKIRELSDYLLQDYPVTVASNLQDEELCGGLWRLVLAQRWMERLKTVAGSKMQGLLERVNTEIHFVTKCAFQPPPSCLRFVQTNISRLLQETSEQLVALKPWITRQNFSRCLELQCQPDSSTLPPPWSPRPLEATAPTAPGGGSGDMARFEDPTRRPYKLPDLCTELNTSLQDIEITCVYCKTVLELTEVFEFAFKDLFVVYRDSIPHAACHKCIDFYSRIRELRYYSDSVMYGPKATLQDIVLHLEPQNEIPVDLLCHEQLSDSEEENDEIDGVNHQHLPARRAEPQRHTMLCMCFYSRIRELRYYSDSVYGDTLEKLTNTGLYNLLIRCLRCQKPLNPAEKLRHLNEKRRFHKIAGHYRGQCHSCCNRARQERLQRRRETQVARRAEPQRHTMLCMCCKCEARIELVVESSADDLRAFQQLFLSTLSFVCPWCASQQMHQKRTAMFQDPQERPRKLPHLCTELQTTIHDIILECVYCKQQLLRREVYDFAFRDLCIVYRDGNPYAVCDKCLKFYSKISEYRYMHGDTPTLHEYMLDLQPETTDLYCYEQLNDSSEEEDEIDGPAGQAEPDRAHYNIVTFCCKCDSTLDKCLKFYSKISEYRYYCYSVYGTTLEQQYNKPLCDLLIRCINCQKPLCPEEKQRHLDKKQRFHNIRGRWTGRCMSCCRSSRTRRETQLHYNIVTFCCKCDSTLRLCVQSTHVDIRTLEDLLMGTLGIVCPICSQKP

SEQ ID NO: 19 - protein, 777 aa, synthetic construct
MDAMKRGLCCVLLLCGAVFVSPSITQDCSFQHSPISSDFAVKIRELSDYLLQDYPVTVASNLQDEELCGGLWRLVLAQRWMERLKTVAGSKMQGLLERVNTEIHFVTKCAFQPPPSCLRFVQTNISRLLQETSEQLVALKPWITRQNFSRCLELQCQPDSSTLPPPWSPRPLEATAPTAPGGGSGDMHQKRTAMFQDPQERPRKLPHLCTELQTTIHDIILECVYCKQQLLRREVYDFAFRDLCIVYRDGNPYAVCDKCLKFYSKISEYRYAAMHGDTPTLHEYMLDLQPETTDLYCYEQLNDSSEEEDEIDGPAGQAEPDRAHYNIVTFCCKCDSTLAADKCLKFYSKISEYRYYCYSVYGTTLEQQYNKPLCDLLIRCINCQKPLCPEEKQRHLDKKQRFHNIRGRWTGRCMSCCRSSRTRRETQLAAHYNIVTFCCKCDSTLRLCVQSTHVDIRTLEDLLMGTLGIVCPICSQKPMARFEDPTRRPYKLPDLCTELNTSLQDIEITCVYCKTVLELTEVFEFAFKDLFVVYRDSIPHAACHKCIDFYSRIRELRYYSDSVAAMYGPKATLQDIVLHLEPQNEIPVDLLCHEQLSDSEEENDEIDGVNHQHLPARRAEPQRHTMLCMCAAFYSRIRELRYYSDSVYGDTLEKLTNTGLYNLLIRCLRCQKPLNPAEKLRHLNEKRRFHKIAGHYRGQCHSCCNRARQERLQRRRETQVAAARRAEPQRHTMLCMCCKCEARIELVVESSADDLRAFQQLFLSTLSFVCPWCASQQ

SEQ ID NO: 20 - protein, 1071 aa, synthetic construct
MDAMKRGLCCVLLLCGAVFVSPSITQDCSFQHSPISSDFAVKIRELSDYLLQDYPVTVASNLQDEELCGGLWRLVLAQRWMERLKTVAGSKMQGLLERVNTEIHFVTKCAFQPPPSCLRFVQTNISRLLQETSEQLVALKPWITRQNFSRCLELQCQPDSSTLPPPWSPRPLEATAPTAPGGGSGDMNVCQDKILEHYENDSKDILEHYENDSKDLCDHICDHIDYWKHIRLECAIMYKARIRLECAIMYKAREMGFHQFDGDICNTMHYTNWIYICEDAQCTVVEGQVDKKWEVHAGGQVILCPESGQRRIKRPRSENCHPNKLLILKCLRYRFKKHCKLSSTWHWTCHDGKHKWHWTCHDGKHKNAIVTLTYDHIDYWKAIRQENAIFFAARHQVVPALNICKAKACKAIEWNTEPKHCFKKGGQHIEVWFDYVAWDSVYYCGDDGWCKTEAEKYGCKGTWEVHFGNSIDCNDSMCSTFDDNVSATELVKMHQKRTAMFQDPQERPRKLPHLCTELQTTIHDIILECVYCKQQLLRREVYDFAFRDLCIVYRDGNPYAVCDKCLKFYSKISEYRYMHGDTPTLHEYMLDLQPETTDLYCYEQLNDSSEEEDEIDGPAGQAEPDRAHYNIVTFCCKCDSTLDKCLKFYSKISEYRYYCYSVYGTTLEQQYNKPLCDLLIRCINCQKPLCPEEKQRHLDKKQRFHNIRGRWTGRCMSCCRSSRTRRETQLHYNIVTFCCKCDSTLRLCVQSTHVDIRTLEDLLMGTLGIVCPICSQKPMARFEDPTRRPYKLPDLCTELNTSLQDIEITCVYCKTVLELTEVFEFAFKDLFVVYRDSIPHAACHKCIDFYSRIRELRYYSDSVMYGPKATLQDIVLHLEPQNEIPVDLLCHEQLSDSEEENDEIDGVNHQHLPARRAEPQRHTMLCMCFYSRIRELRYYSDSVYGDTLEKLTNTGLYNLLIRCLRCQKPLNPAEKLRHLNEKRRFHKIAGHYRGQCHSCCNRARQERLQRRRETQVARRAEPQRHTMLCMCCKCEARIELVVESSADDLRAFQQLFLSTLSFVCPWCASQQ

SEQ ID NO: 21 - protein, 1071 aa, synthetic construct
MDAMKRGLCCVLLLCGAVFVSPSITQDCSFQHSPISSDFAVKIRELSDYLLQDYPVTVASNLQDEELCGGLWRLVLAQRWMERLKTVAGSKMQGLLERVNTEIHFVTKCAFQPPPSCLRFVQTNISRLLQETSEQLVALKPWITRQNFSRCLELQCQPDSSTLPPPWSPRPLEATAPTAPGGGSGDMNVCQDKILEHYENDSKDILEHYENDSKDLCDHICDHIDYWKHIRLECAIMYKARIRLECAIMYKAREMGFHQFDGDICNTMHYTNWIYICEDAQCTVVEGQVDKKWEVHAGGQVILCPESGQRRIKRPRSENCHPNKLLILKCLRYRFKKHCKLSSTWHWTCHDGKHKWHWTCHDGKHKNAIVTLTYDHIDYWKAIRQENAIFFAARHQVVPALNICKAKACKAIEWNTEPKHCFKKGGQHIEVWFDYVAWDSVYYCGDDGWCKTEAEKYGCKGTWEVHFGNSIDCNDSMCSTFDDNVSATELVKMARFEDPTRRPYKLPDLCTELNTSLQDIEITCVYCKTVLELTEVFEFAFKDLFVVYRDSIPHAACHKCIDFYSRIRELRYYSDSVMYGPKATLQDIVLHLEPQNEIPVDLLCHEQLSDSEEENDEIDGVNHQHLPARRAEPQRHTMLCMCFYSRIRELRYYSDSVYGDTLEKLTNTGLYNLLIRCLRCQKPLNPAEKLRHLNEKRRFHKIAGHYRGQCHSCCNRARQERLQRRRETQVARRAEPQRHTMLCMCCKCEARIELVVESSADDLRAFQQLFLSTLSFVCPWCASQQMHQKRTAMFQDPQERPRKLPHLCTELQTTIHDIILECVYCKQQLLRREVYDFAFRDLCIVYRDGNPYAVCDKCLKFYSKISEYRYMHGDTPTLHEYMLDLQPETTDLYCYEQLNDSSEEEDEIDGPAGQAEPDRAHYNIVTFCCKCDSTLDKCLKFYSKISEYRYYCYSVYGTTLEQQYNKPLCDLLIRCINCQKPLCPEEKQRHLDKKQRFHNIRGRWTGRCMSCCRSSRTRRETQLHYNIVTFCCKCDSTLRLCVQSTHVDIRTLEDLLMGTLGIVCPICSQKP

SEQ ID NO: 22 - RNA, 50 nt, synthetic construct
  source 1..50: mol_type = other RNA
acatttgcttctgacacaactgtgttcactagcaacctcaaacagacacc

SEQ ID NO: 23 - RNA, 214 nt, synthetic construct
  source 1..214: mol_type = other RNA
gctcgctttcttgctgtccaatttctattaaaggttcctttgttccctaagtccaactactaaactgggggatattatgaagggccttgagcatctggattctgcctgctcgctttcttgctgtccaatttctattaaaggttcctttgttccctaagtccaactactaaactgggggatattatgaagggccttgagcatctggattctgcct

SEQ ID NO: 24 - RNA, 130 nt, synthetic construct
  source 1..130: mol_type = other RNA
aaaaaaaaaaaaaaaaaaaaaaaaaaaaaaaaaaaaaaaaaaaaaaaaaaaaaaaaaaaagcatatgactaaaaaaaaaaaaaaaaaaaaaaaaaaaaaaaaaaaaaaaaaaaaaaaaaaaaaaaaaaaa

SEQ ID NO: 25 - RNA, 37 nt, synthetic construct
  source 1..37: mol_type = other RNA
actcttctggtccccacagactcagagagaacccacc

SEQ ID NO: 26 - RNA, 110 nt, synthetic construct
  source 1..110: mol_type = other RNA
gctggagcctcggtggccatgcttcttgccccttgggcctccccccagcccctcctccccttcctgcacccgtacccccgtggtctttgaataaagtctgagtgggcggc

SEQ ID NO: 27 - RNA, 123 nt, synthetic construct
  source 1..123: mol_type = other RNA
aaaaaaaaaaaaaaaaaaaaaaaaaaaaaaaaaaaaaaaaaaaaaaaaaaaaaaaaaaaagatatcaaaaaaaaaaaaaaaaaaagaaaaaaaaaaaaaaaaaaagaaaaaaaaaaaaaaaaa

SEQ ID NO: 28 - RNA, 69 nt, synthetic construct
  source 1..69: mol_type = other RNA
atggacgccatgaagcgcggtctttgctgcgtcctgctgttatgcggcgctgtgttcgtcagccctagc

SEQ ID NO: 29 - RNA, 489 nt, synthetic construct
  source 1..489: mol_type = other RNA
ataacgcaggactgcagcttccagcacagccctatatcttcggacttcgcggtcaagattcgggagctctccgactatctgctccaggactatcccgtcacggtcgccagcaaccttcaggacgaagagttgtgtggcggcctgtggcggttagtcctggcgcagcgttggatggagcgcctgaagaccgtggctggttcgaagatgcagggcttgctggagcgggtgaacacggagattcacttcgtgaccaagtgcgcgtttcagcctccgccgagctgtctgaggttcgtgcagacgaacatcagtcggctcttgcaggagactagcgagcagttggtcgcgttgaagccgtggatcacccgccagaacttctcacgttgccttgagctgcagtgccagccggattcctcgaccctccctccgccgtggtcgccgcggccgctggaggccacggcgcccacggcgcctggcggcgggagcggagat

SEQ ID NO: 30 - RNA, 255 nt, synthetic construct
  source 1..255: mol_type = other RNA
atgcatcagaagagaaccgccatgttccaagatccgcaagagagacctagaaaactccctcatctgtgcaccgaactgcagaccaccatccacgacatcatcctggagtgcgtgtattgcaaacaacagctgctgagaagagaggtgtacgacttcgccttcagagacctgtgcatcgtgtaccgggacggcaatccctacgccgtgtgcgacaagtgcctcaagttctatagcaagatcagcgagtatagatac

SEQ ID NO: 31 - RNA, 195 nt, synthetic construct
  source 1..195: mol_type = other RNA
atgcacggagatacgccgaccctgcacgagtacatgctggacctgcagcccgagaccaccgacctgtactgctacgagcagctgaacgacagcagcgaagaggaggacgagattgacggcccggccggccaagccgagcccgacagagcccactacaacatcgtgaccttctgctgtaaatgcgatagcacactg

SEQ ID NO: 32 - RNA, 264 nt, synthetic construct
  source 1..264: mol_type = other RNA
gacaagtgcctgaagttctacagcaagattagcgagtacagatattactgctactccgtgtacgggacaaccctggagcagcagtacaacaagcctctgtgcgacctgctgatccggtgtattaactgtcagaagcccttgtgtcccgaggagaagcagagacacctggacaagaagcagagattccacaacatcagaggcagatggaccggcagatgcatgagctgctgcagaagcagcagaacaagaagagagacacaactg

SEQ ID NO: 33 - RNA, 150 nt, synthetic construct
  source 1..150: mol_type = other RNA
cactacaatatcgtcaccttctgctgcaagtgcgactccacactgcggctctgcgtgcagagcacccacgtggacatcagaaccctggaggacctgctgatgggcaccctgggcatcgtgtgtcccatctgcagccaaaagccctgatga

SEQ ID NO: 34 - RNA, 255 nt, synthetic construct
  source 1..255: mol_type = other RNA
atggcccgattcgaagatcccacaagaagaccctacaagctgcccgacctgtgcaccgagctgaacacaagcctccaagacatcgagattacctgcgtgtactgcaagaccgtgctggagctgaccgaggtgttcgagttcgccttcaaggacctgttcgtggtgtacagagacagcatcccacacgccgcctgccacaagtgcatcgacttctacagccggattcgggaactgcggtactacagcgacagcgtg

SEQ ID NO: 35 - RNA, 195 nt, synthetic construct
  source 1..195: mol_type = other RNA
atgtatgggcccaaggccaccctgcaagacatcgtgctgcacctggagcctcagaacgaaatacccgtggacctgctgtgccatgagcaactgagcgacagcgaggaagagaatgatgagatcgacggcgtgaatcatcagcacctgcccgctagaagggccgagccacaacggcacaccatgctgtgcatgtgc

SEQ ID NO: 36 - RNA, 264 nt, synthetic construct
  source 1..264: mol_type = other RNA
ttctacagcagaatcagagaactccggtattacagcgactccgtgtacggagataccctcgagaagctgaccaacaccggcctgtacaatctgctgatcagatgtctgagatgtcagaaacccttaaatcccgccgagaagctgagacacctgaacgagaagagaagattccacaagatcgccggccactacagagggcagtgccacagctgctgcaacagagctagacaagagagactgcagagaagacgggagacccaagtg

SEQ ID NO: 37 - RNA, 165 nt, synthetic construct
  source 1..165: mol_type = other RNA
gctagaagggctgagccgcaaagacataccatgctgtgtatgtgctgcaaatgcgaggctagaatcgagctggtggtggagagcagcgccgacgacctgagagcctttcagcagctgttcctgagcaccctgagcttcgtgtgtccctggtgcgctagccaacag

SEQ ID NO: 38 - RNA, 918 nt, synthetic construct
  source 1..918: mol_type = other RNA
atgaacgtgtgccaggataagatcttggagcattacgagaatgactccaaggatatcctggagcactatgagaacgactccaaggatctatgtgatcacatctgtgatcacatagattattggaagcacatccggctggagtgcgccattatgtataaggctcggatacggctggaatgtgctataatgtataaagcccgtgagatgggctttcaccagttcgatggtgacatttgtaacacaatgcactatacgaactggatatacatctgcgaggacgcgcagtgtacggtagttgagggtcaggtagacaagaagtgggaggttcacgcgggtgggcaggtcatcctctgcccggagtccgggcagaggaggatcaagcgtccgcggagtgaaaactgccaccctaacaagctactgatcctcaagtgccttcgctatcgcttcaagaagcattgcaagttgtcgtccacgtggcactggacttgccacgacggcaagcacaagtggcactggacgtgccacgacggcaagcacaagaacgcgatagtgacgcttacctatgatcacatagattattggaaagcgatccggcaggagaatgcgatattcttcgctgctagacaccaggtggtgcccgcgttgaatatctgcaaggcgaaggcctgcaaggccatagagtggaacacagagccgaagcactgctttaagaaaggcggtcagcacatcgaggtctggttcgactatgtggcctgggactcggtctactattgcggcgacgacggttggtgcaagaccgaggccgagaaatacggctgcaaagggacgtgggaagttcacttcgggaactccatcgattgcaacgactccatgtgcagcacgtttgacgataacgtgtctgccacggagttggtaaag

SEQ ID NO: 39 - RNA, 1740 nt, synthetic construct
  source 1..1740: mol_type = other RNA
atgcaccagaagagaaccgccatgttccaggaccctcaggagagacctaggaagctgcctcacctgtgtacagagctccagacaaccatccacgacatcatcctggagtgcgtgtactgtaagcagcagctgctgagaagagaggtgtacgacttcgccttcagagacctgtgcatcgtgtacagagacggcaacccttacgccgtgtgcgataagtgtctgaagttctattccaaaatctccgaatataggtacatgcacggcgacacccctaccctgcacgagtacatgctggacctccagcctgagaccacagacctgtactgctacgagcagctgaacgacagctctgaggaagaggacgagattgacggacctgctggccaggccgagcctgacagagcccactacaatatcgtgacattctgttgcaaatgcgactccacactggacaagtgcctgaagttctacagcaagatctctgagtacagatactactgctactctgtgtacggcaccacactggagcagcagtacaacaagcctctgtgcgacctcctgatccgctgcatcaactgccagaagcctctgtgccctgaggagaagcagagacacctggacaagaagcagcggttccacaacatcagaggcagatggaccggcaggtgcatgtcctgctgtagatcctccagaaccagacgggagacccagctgcactacaacatcgtgaccttctgctgcaagtgcgactctaccctgagactgtgcgtgcagtctacccacgtggacatcagaaccctggaggacctgctgatgggcaccctgggcatcgtgtgccctatctgctctcagaagcctatggccaggttcgaggaccctaccagaagaccctacaagctgcctgacctgtgcaccgagctgaacacctctctgcaagacatcgagatcacctgcgtgtactgcaagaccgtgctggagctgaccgaggtgttcgagttcgccttcaaggacctgttcgtggtgtacagagacagcatccctcacgctgcctgccacaagtgcatcgacttctattccaggatcagggagctgcgctattactccgactctgtgatgtacggccccaaggccaccctccaggacatcgtgctgcacctggagcctcagaacgagatccccgtggacctgctgtgccacgagcagctgtctgactctgaagaggagaacgacgagatcgacggcgtgaaccaccagcacctgcctgccaggagagctgaaccccagcggcataccatgctgtgtatgtgcttctactctaggatcagagagctgaggtactactctgactctgtgtacggcgacaccctggagaagctgaccaacaccggcctgtacaacctgctgatccggtgcctgaggtgccagaagcctctgaaccctgccgagaagctgagacacctgaacgagaagagaagattccacaagatcgctggccactacagaggccagtgccactcttgctgcaacagagccagacaggagagactccagcggagaagggagacccaggtggccaggagagccgagcctcagagacacaccatgctgtgcatgtgctgcaagtgcgaggccagaatcgagctggtggtggagagctctgccgacgacctgagagccttccagcagctgttcctgtctaccctgagcttcgtgtgcccttggtgcgcctctcagcagtaa

SEQ ID NO: 40 - RNA, 1743 nt, synthetic construct
  source 1..1743: mol_type = other RNA
atggctagattcgaggaccccacaagaagaccctacaagctgcccgacctgtgcaccgaactgaacacaagcctgcaagacatcgagattacctgcgtgtattgcaagaccgtgctggagctgaccgaggtgttcgagttcgccttcaaggacctgttcgtggtgtacagagatagcatcccccacgccgcctgccacaagtgcatcgacttctatagcagaatcagagaactgcggtactacagcgatagcgtgatgtacggccccaaggccaccctccaagacatcgtcctgcacctggagcctcagaatgagatccccgtggacctgctgtgccacgagcagctgagcgacagcgaggaagaaaacgacgagatcgacggcgtcaatcatcagcacctgcccgctagacgggctgagcctcagcggcacaccatgctgtgtatgtgcttctacagcagaattagagagctcagatactacagcgacagcgtgtatggcgacaccctggagaagctgaccaacaccggcctgtacaatctgctgatcagatgcctgagatgtcagaagcccctcaaccccgccgagaagctgagacacctgaacgagaagagaagattccacaagatcgccggccactacagagggcagtgccacagctgctgcaacagagctagacaagagagactgcagagacggcgggaaacccaagtggctagaagggccgagcctcagagacatacaatgctgtgcatgtgctgcaagtgcgaagctagaatcgagctggtggtggagagcagcgccgacgacctgagagcctttcagcagctgttcctgagcaccctgagcttcgtgtgcccctggtgcgctagccaacagatgcatcagaagagaaccgccatgttccaagacccccaagagagacctagaaagctgccccacctgtgtaccgagctgcagacaaccatccacgacatcatcctggagtgcgtgtactgcaagcagcaactgctgagaagagaggtgtacgacttcgccttcagagacctgtgcatcgtgtaccgggacgggaatccctacgccgtgtgcgacaaatgtctcaagttttatagcaagattagcgagtacagatacatgcacggcgacacccccaccctgcacgagtacatgctggacctgcagcccgagaccaccgacctgtactgctacgaacaactgaacgacagctccgaggaagaggacgaaatcgacggccccgccggccaagccgagcccgacagagcccactacaacattgtgacattctgttgcaagtgtgacagcaccctggacaaatgcctgaagttctacagcaagatcagcgagtacagatattactgctacagcgtgtacggcaccaccctggagcagcagtacaacaagcccctgtgtgacctgctgattagatgcatcaactgtcagaagcccctgtgccccgaggagaagcagagacacctggacaagaagcagagattccacaacatcagaggcagatggaccggcagatgcatgagctgctgcagaagcagcagaacaagaagagagacacagctgcactacaatatcgtgaccttttgctgcaagtgcgatagcaccctgcggctgtgcgtgcagagcacccacgtggacatcagaaccctggaggacctgctgatgggcaccctgggcatcgtgtgccccatctgcagccaaaagccctgatga

SEQ ID NO: 41 - RNA, 1743 nt, synthetic construct
  source 1..1743: mol_type = other RNA
atggcgcggttcgaggacccgactcgcaggccgtataagttaccggatctctgtacagagctgaacacgtccttgcaggacatcgaaatcacctgcgtgtactgcaagaccgtcttggagttaacggaggtgttcgagttcgccttcaaggacttgttcgttgtgtacagagattcgatacctcatgcggcctgccacaagtgcatcgatttctattcgcgcattcgagagctgaggtactactcggacagtgtcatgtacgggcctaaggccacgttacaggacattgtcctccacctggaacctcagaatgagattccggtggacctgctctgccatgagcagctctcggactccgaggaagagaacgatgagatcgacggagtgaaccatcagcacctgcccgcgagaagggcagagccacagcgtcacacaatgctgtgtatgtgcttctactcgcggatcagggagctgaggtattactccgactcggtctacggagacaccttagagaagttgacaaacaccggtttgtacaaccttctcataaggtgtctccgttgccaaaagcctctgaatccggcggagaagctgcggcatctcaacgagaagcggcggtttcacaagatcgccgggcactacagaggacagtgccacagctgctgcaaccgcgccagacaggagcggttgcagcggcggcgcgagacccaggttgcccggcgagccgagccgcagcgacatacaatgctttgtatgtgctgcaagtgcgaggctcggatagagcttgtcgtggaatcttctgcggatgacctgcgagcattccagcagctgtttctgagcactctgtcgttcgtgtgcccgtggtgcgcgagccagcagatgcatcagaagcggactgctatgttccaagacccgcaggagaggccacgcaagcttccacatctgtgtacagagctccaaaccaccatccacgacatcatcctggagtgcgtgtactgcaaacagcagctgctgagaagagaggtgtacgacttcgccttcagagacctgtgcatcgtgtacagagatgggaatccctacgccgtgtgcgacaagtgcctgaagttctatagcaagatcagcgagtacagatacatgcatggcgacacacccaccctgcacgagtacatgctggacctgcagcccgagaccaccgacctgtactgctatgagcagctgaacgacagcagcgaagaggaggacgagatcgacggccctgctggccaagccgagcccgacagagcccactataacatcgtcacattctgttgcaaatgtgactccaccctggacaagtgtctgaaattctatagcaagatctccgagtaccggtactactgttacagcgtgtacggcaccacactggagcagcagtacaacaagccgctttgcgatctgctgatccggtgcatcaactgtcagaagcccttgtgtcccgaagagaagcagagacacctggacaagaagcagagattccacaacatcagaggcagatggaccggcagatgcatgagctgctgcagaagcagcagaacccggagagagacccaactccactacaatatcgtgaccttctgttgcaagtgcgatagcaccctgagactgtgcgtgcagagcacccacgtggacatcagaaccctggaggacctgctgatgggcaccctgggcatcgtgtgccctatctgcagccaaaagccctgatga

SEQ ID NO: 42 - RNA, 1743 nt, synthetic construct
  source 1..1743: mol_type = other RNA
atggctagattcgaggaccccacaagaagaccctacaagctgcccgatctctgcacagagctgaacacaagcctgcaagacatcgagatcacctgcgtgtattgcaagaccgtgctggagctgaccgaggtgttcgagttcgccttcaaggacctgttcgtggtgtacagagacagcatcccccacgccgcctgccacaagtgcatcgacttctacagccggatcagagagctccggtactacagcgactccgtgatgtacggccccaaggccaccctccaagacatcgtgctgcacctggagcctcagaacgagatccccgtggacctgctgtgccacgagcagctgagcgacagcgaggaagagaacgacgaaattgacggcgtgaaccatcagcacctgcccgctagacgggccgagcctcagcggcacaccatgctgtgtatgtgcttctacagcagaatcagagaactcagatattactccgactccgtgtacggcgacacactggagaagctgaccaacaccggcctgtacaacctgctgatcagatgcctgagatgtcagaagcctctcaatcccgccgagaagctgagacacctgaacgagaagagaagattccacaagatcgccggccactacagagggcagtgccacagctgctgcaacagagctagacaagagagactgcagagaagacgggagacccaagtggctagaagggccgagcctcagagacacaccatgctgtgcatgtgctgcaagtgcgaagctagaatcgagctggtggtggagagcagcgccgacgacctgagagcctttcagcagctgttcctgagcaccctgagcttcgtgtgcccctggtgcgctagccaacagatgcatcagaagagaaccgccatgttccaagacccccaagagagacctagaaagctgccccacctgtgtacagagctccaaaccaccatccacgacatcatcctggagtgcgtgtactgcaaacagcagctgctgagaagagaggtgtacgacttcgccttcagagacctgtgcatcgtgtacagagatgggaatccctacgccgtgtgcgacaagtgcctgaagttttatagcaagatcagcgagtacagatacatgcatggcgacacccccaccctgcacgagtacatgctggacctgcagcccgagaccaccgacctgtactgctatgagcagctgaacgacagcagcgaagaggaggacgagatcgacggccccgctggccaagccgagcccgacagagcccactataacatcgtcacattctgttgcaaatgtgactccaccctggacaagtgtctgaaattctatagcaagatctccgagtaccggtactactgttacagcgtgtacggcaccacactggagcagcagtacaacaagcccctgtgcgatctgctgatccggtgcatcaactgtcagaagcccctgtgtcccgaagagaagcagagacacctggacaagaagcagagattccacaacatcagaggcagatggaccggcagatgcatgagctgctgcagaagcagcagaacccggagagagacccaactccactacaatatcgtgaccttctgttgcaagtgcgatagcaccctgagactgtgcgtgcagagcacccacgtggacatcagaaccctggaggacctgctgatgggcaccctgggcatcgtgtgccccatctgcagccaaaagccctgatga

SEQ ID NO: 43 - RNA, 1779 nt, synthetic construct
  source 1..1779: mol_type = other RNA
atgcatcagaagagaaccgccatgttccaagacccccaagagagacctagaaagctgccccacctgtgcaccgagctgcagaccaccatccacgacatcatcctggagtgcgtgtactgtaagcagcagctgctgagaagagaggtgtacgacttcgccttcagagacctgtgcatcgtgtatagagacggcaacccctacgccgtgtgcgataagtgcctgaaattctactccaagatcagcgagtacagatacgccgccatgcacggcgacacccccaccctgcacgagtacatgctggacctgcagcccgagaccaccgacctgtactgctacgagcagctgaacgacagctccgaagaggaggacgagatcgacggccccgccggccaagccgagcccgacagagctcactacaatatcgtgacattctgctgcaagtgcgactccacactggctgccgacaagtgcctcaagttttacagcaagatctccgaatacagatactactgctacagcgtgtacgggaccaccctggagcagcagtacaacaaacctctctgcgacctgctgattagatgcattaattgtcagaagcccctgtgccccgaggagaagcagagacacctggacaagaagcagagattccacaacatcagaggcagatggaccggcagatgcatgagctgctgcagaagcagcagaacaagaagagagacacagctggccgctcactacaacatcgtcaccttctgttgtaagtgcgactccaccctgagactgtgcgtgcagagcacccacgtggacatcagaaccctggaggacctgctgatgggcaccctgggcatcgtgtgccccatctgcagccaaaagcccatggctagattcgaggaccccacaagaagaccctacaagctgcccgacctgtgtacagaactgaacacaagcctgcaagacatcgagatcacctgcgtgtactgcaagaccgtgctggagctgaccgaggtgttcgagttcgccttcaaggacctgttcgtggtgtacagagacagcatcccccacgccgcctgccacaagtgcatcgacttctacagcagaattagagaactgcggtactacagcgacagcgtggccgccatgtacggccccaaggccaccctccaagacatcgtgctgcacctcgagcctcagaacgagatccccgtggacctgctgtgccacgaacagctgagcgacagcgaggaagagaacgacgagattgacggcgtgaaccatcagcacctgcccgctcggagagctgagccccaacggcacaccatgctgtgtatgtgtgccgctttctatagcagaatccgggagctgcggtactattccgacagcgtgtacggggacacactggagaagctgaccaacaccggcctgtacaatctgctgatcagatgcctcagatgtcagaaacccctcaaccctgccgagaagctgagacacctgaacgagaagagaagattccacaagatcgccggccactacagagggcagtgccacagctgctgcaacagagctagacaagagagactgcagagacggagagagacccaagtggccgctgctagaagggccgagcctcagagacacacaatgctgtgcatgtgctgcaaatgcgaggctagaatcgagctggtggtggagagcagcgccgacgacctgagagcctttcagcagctgttcctgagcaccctgagcttcgtgtgcccctggtgcgctagccaacagtgatga

SEQ ID NO: 44 - RNA, 2661 nt, synthetic construct
  source 1..2661: mol_type = other RNA
atgaacgtgtgccaagacaagatcctggaacactacgagaatgacagcaaagacattctggagcactacgaaaatgattccaaggacctgtgtgaccatatctgtgatcatatcgattattggaagcacatcagactggaatgtgctatcatgtacaaggcccggatcagactggagtgcgccatcatgtacaaggctcgggaaatgggcttccatcagttcgacggcgacatctgcaacaccatgcactacaccaactggatctacatctgcgaggacgctcagtgcaccgtggtggagggccaagtggacaagaagtgggaggtgcacgccggcggccaagtgatcctgtgccctgaaagcgggcagagaagaatcaagagaccccggagcgagaactgccaccccaacaagctgctgatcctgaagtgcctgagatacagattcaagaagcactgcaagctgagcagcacctggcactggacctgccatgatggcaaacacaagtggcactggacctgccacgacggcaagcataagaatgccatcgtgaccctgacctacgaccacatcgattattggaaggccatcagacaagagaacgccatcttcttcgccgctagacaccaagtggtgcccgccctgaacatctgcaaggccaaggcctgcaaggccatcgagtggaacaccgagcccaagcactgcttcaagaagggcgggcagcacatcgaggtgtggttcgactacgtcgcctgggatagcgtgtactactgcggcgacgacggctggtgcaagaccgaggccgagaagtacggctgcaagggcacctgggaggtccacttcggcaacagcatcgactgcaacgacagcatgtgcagcaccttcgacgacaacgtgagcgccaccgagctggtgaagatgcatcagaagagaaccgccatgttccaagacccccaagagagacctagaaaactcccccatctgtgcaccgaactgcagaccaccatccacgacatcatcctggagtgcgtgtattgcaaacaacagctgctgagaagagaggtgtacgacttcgccttcagagacctgtgcatcgtgtaccgggacggcaatccctacgccgtgtgcgacaagtgcctcaagttttatagcaagatcagcgagtatagatacatgcacggggacacccccaccctgcacgagtacatgctggacctgcagcccgagaccaccgacctgtactgctacgagcagctgaacgacagcagcgaagaggaggacgagattgacggccccgccggccaagccgagcccgacagagcccactacaacatcgtgaccttctgctgtaaatgcgatagcacactggacaagtgcctgaagttctacagcaagattagcgagtacagatattactgctactccgtgtacgggacaaccctggagcagcagtacaacaagcctctgtgcgacctgctgatccggtgtattaactgtcagaagcccctgtgccccgaggagaagcagagacacctggacaagaagcagagattccacaacatcagaggcagatggaccggcagatgcatgagctgctgcagaagcagcagaacaagaagagagacacaactgcactacaatatcgtcaccttctgctgcaagtgcgactccacactgcggctctgcgtgcagagcacccacgtggacatcagaaccctggaggacctgctgatgggcaccctgggcatcgtgtgccccatctgcagccaaaagcccatggctagattcgaggaccccacaagaagaccctacaagctgcccgacctgtgcaccgagctgaacacaagcctccaagacatcgagattacctgcgtgtactgcaagaccgtgctggagctgaccgaggtgttcgagttcgccttcaaggacctgttcgtggtgtacagagacagcatcccccacgccgcctgccacaagtgcatcgacttctacagccggattcgggaactgcggtactacagcgacagcgtgatgtatggccccaaggccaccctgcaagacatcgtgctgcacctggagcctcagaacgaaatccccgtggacctgctgtgccatgagcaactgagcgacagcgaggaagagaatgatgagatcgacggcgtgaatcatcagcacctgcccgctagaagggccgagccccaacggcacaccatgctgtgcatgtgcttctacagcagaatcagagaactccggtattacagcgactccgtgtacggggataccctcgagaagctgaccaacaccggcctgtacaatctgctgatcagatgtctgagatgtcagaaacccctgaaccccgccgagaagctgagacacctgaacgagaagagaagattccacaagatcgccggccactacagagggcagtgccacagctgctgcaacagagctagacaagagagactgcagagaagacgggagacccaagtggctagaagggctgagccccaaagacataccatgctgtgtatgtgctgcaaatgcgaggctagaatcgagctggtggtggagagcagcgccgacgacctgagagcctttcagcagctgttcctgagcaccctgagcttcgtgtgcccctggtgcgctagccaacagtgatga

SEQ ID NO: 45 - RNA, 2661 nt, synthetic construct
  source 1..2661: mol_type = other RNA
atgaacgtgtgccaggataagatcttggagcattacgagaatgactccaaggatatcctggagcactatgagaacgactccaaggatctatgtgatcacatctgtgatcacatagattattggaagcacatccggctggagtgcgccattatgtataaggcgcgtatccggctggaatgtgctataatgtataaagcccgtgagatgggctttcaccagttcgatggtgacatttgtaacacaatgcactatacgaactggatatacatctgcgaggacgcgcagtgtacggtagttgagggtcaggtagacaagaagtgggaggttcacgccggtgggcaggtcatcctctgcccggagtccgggcagaggaggatcaagcgtccgcggagtgaaaactgccaccctaacaagctactgatcctcaagtgccttcgctatcgcttcaagaagcattgcaagttgtcgtccacgtggcactggacttgccacgacggcaagcacaagtggcactggacgtgccacgacggcaagcacaagaacgcgatagtgacgcttacctatgatcacatagattattggaaagcgatccggcaggagaatgcgatattcttcgctgcacgccaccaggtggtgcccgcgttgaatatctgcaaggcgaaggcctgcaaggccatagagtggaacacagagccgaagcactgctttaagaaaggcggtcagcacatcgaggtctggttcgactatgtggcctgggactcggtctactattgcggcgacgacggttggtgcaagaccgaggccgagaaatacggctgcaagggtacgtgggaagttcactttggtaacagcatcgattgcaacgactccatgtgcagcacgtttgacgataacgtgtctgccacggagttggtaaagatgcaccagaagcggaccgcgatgttccaagatcctcaagagagacctagaaaactcccgcatctgtgcaccgaactgcagaccaccatccacgacatcatcctggagtgcgtgtattgcaaacaacagctgctgagaagagaggtgtacgacttcgccttcagagacctgtgcatcgtgtaccgggacggcaatccctacgccgtgtgcgacaagtgcctcaagttctatagcaagatcagcgagtatagatacatgcacggcgacacaccgaccctgcacgagtacatgctggacctgcagcccgagaccaccgacctgtactgctacgagcagctgaacgacagcagcgaagaggaggacgagattgacggccctgccggccaagccgagcccgacagagcccactacaacatcgtgaccttctgctgtaaatgcgatagcacactggacaagtgcctgaagttctacagcaagattagcgagtacagatattactgctactccgtgtacgggacaaccctggagcagcagtacaacaagcctctgtgcgacctgctgatccggtgtattaactgtcagaagccactgtgccctgaggagaagcagagacacctggacaagaagcagagattccacaacatcagaggcagatggaccggcagatgcatgagctgctgcagaagcagcagaacaagaagagagacacaactgcactacaatatcgtcaccttctgctgcaagtgcgactccacactgcggctctgcgtgcagagcacccacgtggacatcagaaccctggaggacctgctgatgggcaccctgggcatcgtgtgcccgatctgcagccaaaagcccatggctagatttgaagatcccacaagaagaccctacaagctgcccgacctgtgcaccgagctgaacacaagcctccaagacatcgagattacctgcgtgtactgcaagaccgtgctggagctgaccgaggtgttcgagttcgccttcaaggacctgttcgtggtgtacagagacagcattcctcacgccgcctgccacaagtgcatcgacttctacagccggattcgggaactgcggtactacagcgacagcgtgatgtatggcccgaaggccaccctgcaagacatcgtgctgcacctggagcctcagaacgaaatacccgtggacctgctgtgccatgagcaactgagcgacagcgaggaagagaatgatgagatcgacggcgtgaatcatcagcacctgcccgctagaagggccgagccgcaacggcacaccatgctgtgcatgtgcttctacagcagaatcagagaactccggtattacagcgactccgtgtacggagacaccctcgagaagctgaccaacaccggcctgtacaatctgctgatcagatgtctgagatgtcagaaacccttgaatcccgccgagaagctgagacacctgaacgagaagagaagattccacaagatcgccggccactacagagggcagtgccacagctgctgcaacagagctagacaagagagactgcagagaagacgggagacccaagtggctagaagggctgagcctcaaagacataccatgctgtgtatgtgctgcaaatgcgaggctagaatcgagctggtggtggagagcagcgccgacgacctgagagcctttcagcagctgttcctgagcaccctgagcttcgtgtgtccctggtgcgctagccaacagtgatga

SEQ ID NO: 46 - RNA, 2661 nt, synthetic construct
  source 1..2661: mol_type = other RNA
atgaacgtgtgccaggataagatcttggagcattacgagaatgactccaaggatatcctggagcactatgagaacgactccaaggatctatgtgatcacatctgtgatcacatagattattggaagcacatccggctggagtgcgccattatgtataaggctcggatacggctggaatgtgctataatgtataaagcccgtgagatgggctttcaccagttcgatggtgacatttgtaacacaatgcactatacgaactggatatacatctgcgaggacgcgcagtgtacggtagttgagggtcaggtagacaagaagtgggaggttcacgcgggtgggcaggtcatcctctgcccggagtccgggcagaggaggatcaagcgtccgcggagtgaaaactgccaccctaacaagctactgatcctcaagtgccttcgctatcgcttcaagaagcattgcaagttgtcgtccacgtggcactggacttgccacgacggcaagcacaagtggcactggacgtgccacgacggcaagcacaagaacgcgatagtgacgcttacctatgatcacatagattattggaaagcgatccggcaggagaatgcgatattcttcgctgctagacaccaggtggtgcccgcgttgaatatctgcaaggcgaaggcctgcaaggccatagagtggaacacagagccgaagcactgctttaagaaaggcggtcagcacatcgaggtctggttcgactatgtggcctgggactcggtctactattgcggcgacgacggttggtgcaagaccgaggccgagaaatacggctgcaaagggacgtgggaagttcacttcgggaactccatcgattgcaacgactccatgtgcagcacgtttgacgataacgtgtctgccacggagttggtaaagatggcccgattcgaagatcccacaagaagaccctacaagctgcccgacctgtgcaccgagctgaacacaagcctccaagacatcgagattacctgcgtgtactgcaagaccgtgctggagctgaccgaggtgttcgagttcgccttcaaggacctgttcgtggtgtacagagacagcatcccacacgccgcctgccacaagtgcatcgacttctacagccggattcgggaactgcggtactacagcgacagcgtgatgtatgggcccaaggccaccctgcaagacatcgtgctgcacctggagcctcagaacgaaatacccgtggacctgctgtgccatgagcaactgagcgacagcgaggaagagaatgatgagatcgacggcgtgaatcatcagcacctgcccgctagaagggccgagccacaacggcacaccatgctgtgcatgtgcttctacagcagaatcagagaactccggtattacagcgactccgtgtacggagataccctcgagaagctgaccaacaccggcctgtacaatctgctgatcagatgtctgagatgtcagaaacccttaaatcccgccgagaagctgagacacctgaacgagaagagaagattccacaagatcgccggccactacagagggcagtgccacagctgctgcaacagagctagacaagagagactgcagagaagacgggagacccaagtggctagaagggctgagccgcaaagacataccatgctgtgtatgtgctgcaaatgcgaggctagaatcgagctggtggtggagagcagcgccgacgacctgagagcctttcagcagctgttcctgagcaccctgagcttcgtgtgtccctggtgcgctagccaacagatgcatcagaagagaaccgccatgttccaagatccgcaagagagacctagaaaactccctcatctgtgcaccgaactgcagaccaccatccacgacatcatcctggagtgcgtgtattgcaaacaacagctgctgagaagagaggtgtacgacttcgccttcagagacctgtgcatcgtgtaccgggacggcaatccctacgccgtgtgcgacaagtgcctcaagttctatagcaagatcagcgagtatagatacatgcacggagatacgccgaccctgcacgagtacatgctggacctgcagcccgagaccaccgacctgtactgctacgagcagctgaacgacagcagcgaagaggaggacgagattgacggcccggccggccaagccgagcccgacagagcccactacaacatcgtgaccttctgctgtaaatgcgatagcacactggacaagtgcctgaagttctacagcaagattagcgagtacagatattactgctactccgtgtacgggacaaccctggagcagcagtacaacaagcctctgtgcgacctgctgatccggtgtattaactgtcagaagcccttgtgtcccgaggagaagcagagacacctggacaagaagcagagattccacaacatcagaggcagatggaccggcagatgcatgagctgctgcagaagcagcagaacaagaagagagacacaactgcactacaatatcgtcaccttctgctgcaagtgcgactccacactgcggctctgcgtgcagagcacccacgtggacatcagaaccctggaggacctgctgatgggcaccctgggcatcgtgtgtcccatctgcagccaaaagccctgatga

SEQ ID NO: 47 - RNA, 2298 nt, synthetic construct
  source 1..2298: mol_type = other RNA
atggatgctatgaaacggggcctgtgctgcgtgctgctcctgtgcggcgctgtgtttgtgagccctagcatcacccaggactgctccttccaacacagccccatctcctccgacttcgctgtcaaaatccgtgagctgtctgactacctgcttcaagattacccagtcaccgtggcctccaacctgcaggacgaggagctctgcgggggcctctggcggctggtcctggcacagcgctggatggagcggctcaagactgtcgctgggtccaagatgcaaggcttgctggagcgcgtgaacacggagatacactttgtcaccaaatgtgcctttcagcccccccccagctgtcttcgcttcgtccagaccaacatctcccgcctcctgcaggagacctccgagcagctggtggcgctgaagccctggatcactcgccagaacttctcccggtgcctggagctgcagtgtcagcccgactcctcaaccctgccacccccatggagtccccggcccctggaggccacagccccgacagccccgggcggcggcagcggcgatatgcaccagaagagaaccgccatgttccaggaccctcaggagagacctaggaagctgcctcacctgtgtacagagctccagacaaccatccacgacatcatcctggagtgcgtgtactgtaagcagcagctgctgagaagagaggtgtacgacttcgccttcagagacctgtgcatcgtgtacagagacggcaacccttacgccgtgtgcgataagtgtctgaagttctattccaaaatctccgaatataggtacatgcacggcgacacccctaccctgcacgagtacatgctggacctccagcctgagaccacagacctgtactgctacgagcagctgaacgacagctctgaggaagaggacgagattgacggacctgctggccaggccgagcctgacagagcccactacaatatcgtgacattctgttgcaaatgcgactccacactggacaagtgcctgaagttctacagcaagatctctgagtacagatactactgctactctgtgtacggcaccacactggagcagcagtacaacaagcctctgtgcgacctcctgatccgctgcatcaactgccagaagcctctgtgccctgaggagaagcagagacacctggacaagaagcagcggttccacaacatcagaggcagatggaccggcaggtgcatgtcctgctgtagatcctccagaaccagacgggagacccagctgcactacaacatcgtgaccttctgctgcaagtgcgactctaccctgagactgtgcgtgcagtctacccacgtggacatcagaaccctggaggacctgctgatgggcaccctgggcatcgtgtgccctatctgctctcagaagcctatggccaggttcgaggaccctaccagaagaccctacaagctgcctgacctgtgcaccgagctgaacacctctctgcaagacatcgagatcacctgcgtgtactgcaagaccgtgctggagctgaccgaggtgttcgagttcgccttcaaggacctgttcgtggtgtacagagacagcatccctcacgctgcctgccacaagtgcatcgacttctattccaggatcagggagctgcgctattactccgactctgtgatgtacggccccaaggccaccctccaggacatcgtgctgcacctggagcctcagaacgagatccccgtggacctgctgtgccacgagcagctgtctgactctgaagaggagaacgacgagatcgacggcgtgaaccaccagcacctgcctgccaggagagctgaaccccagcggcataccatgctgtgtatgtgcttctactctaggatcagagagctgaggtactactctgactctgtgtacggcgacaccctggagaagctgaccaacaccggcctgtacaacctgctgatccggtgcctgaggtgccagaagcctctgaaccctgccgagaagctgagacacctgaacgagaagagaagattccacaagatcgctggccactacagaggccagtgccactcttgctgcaacagagccagacaggagagactccagcggagaagggagacccaggtggccaggagagccgagcctcagagacacaccatgctgtgcatgtgctgcaagtgcgaggccagaatcgagctggtggtggagagctctgccgacgacctgagagccttccagcagctgttcctgtctaccctgagcttcgtgtgcccttggtgcgcctctcagcagtaa

SEQ ID NO: 48 - RNA, 2301 nt, synthetic construct
  source 1..2301: mol_type = other RNA
atggacgccatgaagagaggcctgtgctgcgtgctgctcctgtgcggcgccgtgttcgtgagccctagcatcacccaagactgcagctttcagcacagccccatcagcagcgacttcgccgtgaagatcagagagctgagcgactacctgctgcaagactaccccgtgaccgtggctagcaacctgcaagacgaggagctgtgcggcggcctgtggagactggtgctggctcagagatggatggagagactgaagaccgtggccggcagcaagatgcaaggcctgctggagagagtgaacaccgagatccacttcgtgaccaagtgcgcctttcagccccctcctagctgcctgagattcgtgcagaccaacatcagcagactgctgcaagagacaagcgagcagctggtggccctgaagccctggatcacaagacagaacttcagcagatgcctcgagctgcagtgtcagcctgacagctccaccctgcctcctccctggtcccctagacccctggaggctaccgctcccaccgcccccggcgggggcagcggcgacatggctagattcgaggaccccacaagaagaccctacaagctgcccgacctgtgcaccgaactgaacacaagcctgcaagacatcgagattacctgcgtgtattgcaagaccgtgctggagctgaccgaggtgttcgagttcgccttcaaggacctgttcgtggtgtacagagatagcatcccccacgccgcctgccacaagtgcatcgacttctatagcagaatcagagaactgcggtactacagcgatagcgtgatgtacggccccaaggccaccctccaagacatcgtcctgcacctggagcctcagaatgagatccccgtggacctgctgtgccacgagcagctgagcgacagcgaggaagaaaacgacgagatcgacggcgtcaatcatcagcacctgcccgctagacgggctgagcctcagcggcacaccatgctgtgtatgtgcttctacagcagaattagagagctcagatactacagcgacagcgtgtatggcgacaccctggagaagctgaccaacaccggcctgtacaatctgctgatcagatgcctgagatgtcagaagcccctcaaccccgccgagaagctgagacacctgaacgagaagagaagattccacaagatcgccggccactacagagggcagtgccacagctgctgcaacagagctagacaagagagactgcagagacggcgggaaacccaagtggctagaagggccgagcctcagagacatacaatgctgtgcatgtgctgcaagtgcgaagctagaatcgagctggtggtggagagcagcgccgacgacctgagagcctttcagcagctgttcctgagcaccctgagcttcgtgtgcccctggtgcgctagccaacagatgcatcagaagagaaccgccatgttccaagacccccaagagagacctagaaagctgccccacctgtgtaccgagctgcagacaaccatccacgacatcatcctggagtgcgtgtactgcaagcagcaactgctgagaagagaggtgtacgacttcgccttcagagacctgtgcatcgtgtaccgggacgggaatccctacgccgtgtgcgacaaatgtctcaagttttatagcaagattagcgagtacagatacatgcacggcgacacccccaccctgcacgagtacatgctggacctgcagcccgagaccaccgacctgtactgctacgaacaactgaacgacagctccgaggaagaggacgaaatcgacggccccgccggccaagccgagcccgacagagcccactacaacattgtgacattctgttgcaagtgtgacagcaccctggacaaatgcctgaagttctacagcaagatcagcgagtacagatattactgctacagcgtgtacggcaccaccctggagcagcagtacaacaagcccctgtgtgacctgctgattagatgcatcaactgtcagaagcccctgtgccccgaggagaagcagagacacctggacaagaagcagagattccacaacatcagaggcagatggaccggcagatgcatgagctgctgcagaagcagcagaacaagaagagagacacagctgcactacaatatcgtgaccttttgctgcaagtgcgatagcaccctgcggctgtgcgtgcagagcacccacgtggacatcagaaccctggaggacctgctgatgggcaccctgggcatcgtgtgccccatctgcagccaaaagccctgatga

SEQ ID NO: 49 - RNA, 2301 nt, synthetic construct
  source 1..2301: mol_type = other RNA
atggacgccatgaagcgcgggctttgctgcgtcctgctgttatgcggcgctgtgttcgtcagccctagcataacgcaggactgcagcttccagcacagccctatatcttcggacttcgcggtcaagattcgggagctctccgactatctgctccaggactatcccgtcacggtcgccagcaaccttcaggacgaagagttgtgtggcggcctgtggcggttagtcctggcgcagcgttggatggagcgcctgaagaccgtggctggttcgaagatgcagggcttgctggagcgggtgaacacggagattcacttcgtgaccaagtgcgcgtttcagcctccgccgagctgtctgaggttcgtgcagacgaacatcagtcggctcttgcaggagactagcgagcagttggtcgcgttgaagccgtggatcacccgccagaactttagtcggtgcctcgagctgcagtgccagccagattcctcgaccctccctccgccgtggtcgccgcggccgctggaggccacggcgcccacggcgcctggcggcgggagcggtgacatggcgcggttcgaggacccgactcgcaggccgtataagttaccggatctctgtacagagctgaacacgtccttgcaggacatcgaaatcacctgcgtgtactgcaagaccgtcttggagttaacggaggtgttcgagttcgccttcaaggacttgttcgttgtgtacagagattcgatacctcatgcggcctgccacaagtgcatcgatttctattcgcgcattcgagagctgaggtactactcggacagtgtcatgtacgggcctaaggccacgttacaggacattgtcctccacctggaacctcagaatgagattccggtggacctgctctgccatgagcagctctcggactccgaggaagagaacgatgagatcgacggagtgaaccatcagcacctgcccgcgagaagggcagagccacagcgtcacacaatgctgtgtatgtgcttctactcgcggatcagggagctgaggtattactccgactcggtctacggagacaccttagagaagttgacaaacaccggtttgtacaaccttctcataaggtgtctccgttgccaaaagcctctgaatccggcggagaagctgcggcatctcaacgagaagcggcggtttcacaagatcgccgggcactacagaggacagtgccacagctgctgcaaccgcgccagacaggagcggttgcagcggcggcgcgagacccaggttgcccggcgagccgagccgcagcgacatacaatgctttgtatgtgctgcaagtgcgaggctcggatagagcttgtcgtggaatcttctgcggatgacctgcgagcattccagcagctgtttctgagcactctgtcgttcgtgtgcccgtggtgcgcgagccagcagatgcatcagaagcggactgctatgttccaagacccgcaggagaggccacgcaagcttccacatctgtgtacagagctccaaaccaccatccacgacatcatcctggagtgcgtgtactgcaaacagcagctgctgagaagagaggtgtacgacttcgccttcagagacctgtgcatcgtgtacagagatgggaatccctacgccgtgtgcgacaagtgcctgaagttctatagcaagatcagcgagtacagatacatgcatggcgacacacccaccctgcacgagtacatgctggacctgcagcccgagaccaccgacctgtactgctatgagcagctgaacgacagcagcgaagaggaggacgagatcgacggccctgctggccaagccgagcccgacagagcccactataacatcgtcacattctgttgcaaatgtgactccaccctggacaagtgtctgaaattctatagcaagatctccgagtaccggtactactgttacagcgtgtacggcaccacactggagcagcagtacaacaagccgctttgcgatctgctgatccggtgcatcaactgtcagaagcccttgtgtcccgaagagaagcagagacacctggacaagaagcagagattccacaacatcagaggcagatggaccggcagatgcatgagctgctgcagaagcagcagaacccggagagagacccaactccactacaatatcgtgaccttctgttgcaagtgcgatagcaccctgagactgtgcgtgcagagcacccacgtggacatcagaaccctggaggacctgctgatgggcaccctgggcatcgtgtgccctatctgcagccaaaagccctgatga

SEQ ID NO: 50 - RNA, 2301 nt, synthetic construct
  source 1..2301: mol_type = other RNA
atggacgccatgaagagaggcctgtgctgcgtgctgctcctgtgcggcgccgtgttcgtgagccctagcatcacccaagactgcagctttcagcacagccccatcagcagcgacttcgccgtgaagatcagagaactcagcgactacctgctgcaagactaccccgtgaccgtggctagcaacctgcaagacgaggagctgtgcggcggcctgtggagactggtgctggctcagagatggatggagagactgaagaccgtggccggcagcaagatgcaaggcctgctggagagagtgaacaccgagatccacttcgtgaccaagtgcgcctttcagccccctcctagctgcctgagattcgtgcagaccaacatcagcagactgctgcaagagacaagcgagcagctggtggccctgaagccctggatcacaagacagaacttcagcagatgcctggagctgcaatgtcagcccgacagcagcaccctcccccctccctggagccctagacccctcgaagccaccgctcccaccgcccccggcgggggcagcggcgacatggctagattcgaggaccccacaagaagaccctacaagctgcccgatctctgcacagagctgaacacaagcctgcaagacatcgagatcacctgcgtgtattgcaagaccgtgctggagctgaccgaggtgttcgagttcgccttcaaggacctgttcgtggtgtacagagacagcatcccccacgccgcctgccacaagtgcatcgacttctacagccggatcagagagctccggtactacagcgactccgtgatgtacggccccaaggccaccctccaagacatcgtgctgcacctggagcctcagaacgagatccccgtggacctgctgtgccacgagcagctgagcgacagcgaggaagagaacgacgaaattgacggcgtgaaccatcagcacctgcccgctagacgggccgagcctcagcggcacaccatgctgtgtatgtgcttctacagcagaatcagagaactcagatattactccgactccgtgtacggcgacacactggagaagctgaccaacaccggcctgtacaacctgctgatcagatgcctgagatgtcagaagcctctcaatcccgccgagaagctgagacacctgaacgagaagagaagattccacaagatcgccggccactacagagggcagtgccacagctgctgcaacagagctagacaagagagactgcagagaagacgggagacccaagtggctagaagggccgagcctcagagacacaccatgctgtgcatgtgctgcaagtgcgaagctagaatcgagctggtggtggagagcagcgccgacgacctgagagcctttcagcagctgttcctgagcaccctgagcttcgtgtgcccctggtgcgctagccaacagatgcatcagaagagaaccgccatgttccaagacccccaagagagacctagaaagctgccccacctgtgtacagagctccaaaccaccatccacgacatcatcctggagtgcgtgtactgcaaacagcagctgctgagaagagaggtgtacgacttcgccttcagagacctgtgcatcgtgtacagagatgggaatccctacgccgtgtgcgacaagtgcctgaagttttatagcaagatcagcgagtacagatacatgcatggcgacacccccaccctgcacgagtacatgctggacctgcagcccgagaccaccgacctgtactgctatgagcagctgaacgacagcagcgaagaggaggacgagatcgacggccccgctggccaagccgagcccgacagagcccactataacatcgtcacattctgttgcaaatgtgactccaccctggacaagtgtctgaaattctatagcaagatctccgagtaccggtactactgttacagcgtgtacggcaccacactggagcagcagtacaacaagcccctgtgcgatctgctgatccggtgcatcaactgtcagaagcccctgtgtcccgaagagaagcagagacacctggacaagaagcagagattccacaacatcagaggcagatggaccggcagatgcatgagctgctgcagaagcagcagaacccggagagagacccaactccactacaatatcgtgaccttctgttgcaagtgcgatagcaccctgagactgtgcgtgcagagcacccacgtggacatcagaaccctggaggacctgctgatgggcaccctgggcatcgtgtgccccatctgcagccaaaagccctgatga

SEQ ID NO: 51 - RNA, 2337 nt, synthetic construct
  source 1..2337: mol_type = other RNA
atggacgccatgaagagaggcctgtgctgcgtgctgctcctgtgcggcgccgtgttcgtgagccctagcatcacccaagactgcagctttcagcacagccccatcagcagcgacttcgccgtgaagatccgggagctgtccgactacctgctgcaagactaccccgtgaccgtggctagcaacctgcaagacgaggagctgtgcggcggcctgtggagactggtgctggctcagagatggatggagagactgaagaccgtggccggcagcaagatgcaaggcctgctggagagagtgaacaccgagatccacttcgtgaccaagtgcgcctttcagccccctcctagctgcctgagattcgtgcagaccaacatcagcagactgctgcaagagacaagcgagcagctggtggccctgaagccctggatcacaagacagaacttcagcagatgcctggaactccaatgtcagcccgacagcagcaccctgcctcccccctggagccctagacccctcgaagccacagcccccacagcccccggggggggcagcggcgacatgcatcagaagagaaccgccatgttccaagacccccaagagagacctagaaagctgccccacctgtgcaccgagctgcagaccaccatccacgacatcatcctggagtgcgtgtactgtaagcagcagctgctgagaagagaggtgtacgacttcgccttcagagacctgtgcatcgtgtatagagacggcaacccctacgccgtgtgcgataagtgcctgaaattctactccaagatcagcgagtacagatacgccgccatgcacggcgacacccccaccctgcacgagtacatgctggacctgcagcccgagaccaccgacctgtactgctacgagcagctgaacgacagctccgaagaggaggacgagatcgacggccccgccggccaagccgagcccgacagagctcactacaatatcgtgacattctgctgcaagtgcgactccacactggctgccgacaagtgcctcaagttttacagcaagatctccgaatacagatactactgctacagcgtgtacgggaccaccctggagcagcagtacaacaaacctctctgcgacctgctgattagatgcattaattgtcagaagcccctgtgccccgaggagaagcagagacacctggacaagaagcagagattccacaacatcagaggcagatggaccggcagatgcatgagctgctgcagaagcagcagaacaagaagagagacacagctggccgctcactacaacatcgtcaccttctgttgtaagtgcgactccaccctgagactgtgcgtgcagagcacccacgtggacatcagaaccctggaggacctgctgatgggcaccctgggcatcgtgtgccccatctgcagccaaaagcccatggctagattcgaggaccccacaagaagaccctacaagctgcccgacctgtgtacagaactgaacacaagcctgcaagacatcgagatcacctgcgtgtactgcaagaccgtgctggagctgaccgaggtgttcgagttcgccttcaaggacctgttcgtggtgtacagagacagcatcccccacgccgcctgccacaagtgcatcgacttctacagcagaattagagaactgcggtactacagcgacagcgtggccgccatgtacggccccaaggccaccctccaagacatcgtgctgcacctcgagcctcagaacgagatccccgtggacctgctgtgccacgaacagctgagcgacagcgaggaagagaacgacgagattgacggcgtgaaccatcagcacctgcccgctcggagagctgagccccaacggcacaccatgctgtgtatgtgtgccgctttctatagcagaatccgggagctgcggtactattccgacagcgtgtacggggacacactggagaagctgaccaacaccggcctgtacaatctgctgatcagatgcctcagatgtcagaaacccctcaaccctgccgagaagctgagacacctgaacgagaagagaagattccacaagatcgccggccactacagagggcagtgccacagctgctgcaacagagctagacaagagagactgcagagacggagagagacccaagtggccgctgctagaagggccgagcctcagagacacacaatgctgtgcatgtgctgcaaatgcgaggctagaatcgagctggtggtggagagcagcgccgacgacctgagagcctttcagcagctgttcctgagcaccctgagcttcgtgtgcccctggtgcgctagccaacagtgatga

SEQ ID NO: 52 - RNA, 3219 nt, synthetic construct
  source 1..3219: mol_type = other RNA
atggacgccatgaagagaggcctgtgctgcgtgctgctcctgtgcggcgccgtgttcgtgagccctagcatcacccaagactgcagctttcagcacagccccatcagcagcgacttcgccgtgaagatcagagagctgagcgactacctgctgcaagactaccccgtgaccgtggctagcaacctgcaagacgaggagctgtgcggcggcctgtggagactggtgctggctcagagatggatggagagactgaagaccgtggccggcagcaagatgcaaggcctgctggagagagtgaacaccgagatccacttcgtgaccaagtgcgcctttcagccccctcctagctgcctgagattcgtgcagaccaacatcagcagactgctgcaagagacaagcgagcagctggtggccctgaagccctggatcacaagacagaacttcagcagatgcctggagctgcagtgtcagcctgacagcagcaccctcccccctccctggagcccccggcctctggaggctacagcccccacagcccccggcgggggcagcggcgacatgaacgtgtgccaagacaagatcctggaacactacgagaatgacagcaaagacattctggagcactacgaaaatgattccaaggacctgtgtgaccatatctgtgatcatatcgattattggaagcacatcagactggaatgtgctatcatgtacaaggcccggatcagactggagtgcgccatcatgtacaaggctcgggaaatgggcttccatcagttcgacggcgacatctgcaacaccatgcactacaccaactggatctacatctgcgaggacgctcagtgcaccgtggtggagggccaagtggacaagaagtgggaggtgcacgccggcggccaagtgatcctgtgccctgaaagcgggcagagaagaatcaagagaccccggagcgagaactgccaccccaacaagctgctgatcctgaagtgcctgagatacagattcaagaagcactgcaagctgagcagcacctggcactggacctgccatgatggcaaacacaagtggcactggacctgccacgacggcaagcataagaatgccatcgtgaccctgacctacgaccacatcgattattggaaggccatcagacaagagaacgccatcttcttcgccgctagacaccaagtggtgcccgccctgaacatctgcaaggccaaggcctgcaaggccatcgagtggaacaccgagcccaagcactgcttcaagaagggcgggcagcacatcgaggtgtggttcgactacgtcgcctgggatagcgtgtactactgcggcgacgacggctggtgcaagaccgaggccgagaagtacggctgcaagggcacctgggaggtccacttcggcaacagcatcgactgcaacgacagcatgtgcagcaccttcgacgacaacgtgagcgccaccgagctggtgaagatgcatcagaagagaaccgccatgttccaagacccccaagagagacctagaaaactcccccatctgtgcaccgaactgcagaccaccatccacgacatcatcctggagtgcgtgtattgcaaacaacagctgctgagaagagaggtgtacgacttcgccttcagagacctgtgcatcgtgtaccgggacggcaatccctacgccgtgtgcgacaagtgcctcaagttttatagcaagatcagcgagtatagatacatgcacggggacacccccaccctgcacgagtacatgctggacctgcagcccgagaccaccgacctgtactgctacgagcagctgaacgacagcagcgaagaggaggacgagattgacggccccgccggccaagccgagcccgacagagcccactacaacatcgtgaccttctgctgtaaatgcgatagcacactggacaagtgcctgaagttctacagcaagattagcgagtacagatattactgctactccgtgtacgggacaaccctggagcagcagtacaacaagcctctgtgcgacctgctgatccggtgtattaactgtcagaagcccctgtgccccgaggagaagcagagacacctggacaagaagcagagattccacaacatcagaggcagatggaccggcagatgcatgagctgctgcagaagcagcagaacaagaagagagacacaactgcactacaatatcgtcaccttctgctgcaagtgcgactccacactgcggctctgcgtgcagagcacccacgtggacatcagaaccctggaggacctgctgatgggcaccctgggcatcgtgtgccccatctgcagccaaaagcccatggctagattcgaggaccccacaagaagaccctacaagctgcccgacctgtgcaccgagctgaacacaagcctccaagacatcgagattacctgcgtgtactgcaagaccgtgctggagctgaccgaggtgttcgagttcgccttcaaggacctgttcgtggtgtacagagacagcatcccccacgccgcctgccacaagtgcatcgacttctacagccggattcgggaactgcggtactacagcgacagcgtgatgtatggccccaaggccaccctgcaagacatcgtgctgcacctggagcctcagaacgaaatccccgtggacctgctgtgccatgagcaactgagcgacagcgaggaagagaatgatgagatcgacggcgtgaatcatcagcacctgcccgctagaagggccgagccccaacggcacaccatgctgtgcatgtgcttctacagcagaatcagagaactccggtattacagcgactccgtgtacggggataccctcgagaagctgaccaacaccggcctgtacaatctgctgatcagatgtctgagatgtcagaaacccctgaaccccgccgagaagctgagacacctgaacgagaagagaagattccacaagatcgccggccactacagagggcagtgccacagctgctgcaacagagctagacaagagagactgcagagaagacgggagacccaagtggctagaagggctgagccccaaagacataccatgctgtgtatgtgctgcaaatgcgaggctagaatcgagctggtggtggagagcagcgccgacgacctgagagcctttcagcagctgttcctgagcaccctgagcttcgtgtgcccctggtgcgctagccaacagtgatga

SEQ ID NO: 53 - RNA, 3219 nt, synthetic construct
  source 1..3219: mol_type = other RNA
atggacgccatgaagcgcggtctgtgctgcgtcctgctgttatgcggcgctgtgttcgtcagccctagcataacgcaggactgcagcttccagcacagccctatatcttcggacttcgcggtcaagattcgggagctctccgactatctgctccaggactatcccgtcacggtcgccagcaaccttcaggacgaagagttgtgtggcggcctgtggcggttagtcctggcgcagcgttggatggagcgcctgaagaccgtggctggttcgaagatgcagggcttgctggagcgggtgaacacggagattcacttcgtgaccaagtgcgcgtttcagcctccgccgagctgtctgaggttcgtgcagacgaacatcagtcggctcttgcaggagactagcgagcagttggtcgcgttgaagccgtggatcacccgccagaacttctcacgttgccttgagctgcagtgccagccggattcctcgaccctccctccgccgtggtcgccgcggccgctggaggccacggcgcccacggcgcctggcggagggtcgggcgacatgaacgtgtgccaggataagatcttggagcattacgagaatgactccaaggatatcctggagcactatgagaacgactccaaggatctatgtgatcacatctgtgatcacatagattattggaagcacatccggctggagtgcgccattatgtataaggcgcgtatccggctggaatgtgctataatgtataaagcccgtgagatgggctttcaccagttcgatggtgacatttgtaacacaatgcactatacgaactggatatacatctgcgaggacgcgcagtgtacggtagttgagggtcaggtagacaagaagtgggaggttcacgccggtgggcaggtcatcctctgcccggagtccgggcagaggaggatcaagcgtccgcggagtgaaaactgccaccctaacaagctactgatcctcaagtgccttcgctatcgcttcaagaagcattgcaagttgtcgtccacgtggcactggacttgccacgacggcaagcacaagtggcactggacgtgccacgacggcaagcacaagaacgcgatagtgacgcttacctatgatcacatagattattggaaagcgatccggcaggagaatgcgatattcttcgctgcacgccaccaggtggtgcccgcgttgaatatctgcaaggcgaaggcctgcaaggccatagagtggaacacagagccgaagcactgctttaagaaaggcggtcagcacatcgaggtctggttcgactatgtggcctgggactcggtctactattgcggcgacgacggttggtgcaagaccgaggccgagaaatacggctgcaagggtacgtgggaagttcactttggtaacagcatcgattgcaacgactccatgtgcagcacgtttgacgataacgtgtctgccacggagttggtaaagatgcaccagaagcggaccgcgatgttccaagatcctcaagagagacctagaaaactcccgcatctgtgcaccgaactgcagaccaccatccacgacatcatcctggagtgcgtgtattgcaaacaacagctgctgagaagagaggtgtacgacttcgccttcagagacctgtgcatcgtgtaccgggacggcaatccctacgccgtgtgcgacaagtgcctcaagttctatagcaagatcagcgagtatagatacatgcacggcgacacaccgaccctgcacgagtacatgctggacctgcagcccgagaccaccgacctgtactgctacgagcagctgaacgacagcagcgaagaggaggacgagattgacggccctgccggccaagccgagcccgacagagcccactacaacatcgtgaccttctgctgtaaatgcgatagcacactggacaagtgcctgaagttctacagcaagattagcgagtacagatattactgctactccgtgtacgggacaaccctggagcagcagtacaacaagcctctgtgcgacctgctgatccggtgtattaactgtcagaagccactgtgccctgaggagaagcagagacacctggacaagaagcagagattccacaacatcagaggcagatggaccggcagatgcatgagctgctgcagaagcagcagaacaagaagagagacacaactgcactacaatatcgtcaccttctgctgcaagtgcgactccacactgcggctctgcgtgcagagcacccacgtggacatcagaaccctggaggacctgctgatgggcaccctgggcatcgtgtgcccgatctgcagccaaaagcccatggctagatttgaagatcccacaagaagaccctacaagctgcccgacctgtgcaccgagctgaacacaagcctccaagacatcgagattacctgcgtgtactgcaagaccgtgctggagctgaccgaggtgttcgagttcgccttcaaggacctgttcgtggtgtacagagacagcattcctcacgccgcctgccacaagtgcatcgacttctacagccggattcgggaactgcggtactacagcgacagcgtgatgtatggcccgaaggccaccctgcaagacatcgtgctgcacctggagcctcagaacgaaatacccgtggacctgctgtgccatgagcaactgagcgacagcgaggaagagaatgatgagatcgacggcgtgaatcatcagcacctgcccgctagaagggccgagccgcaacggcacaccatgctgtgcatgtgcttctacagcagaatcagagaactccggtattacagcgactccgtgtacggagacaccctcgagaagctgaccaacaccggcctgtacaatctgctgatcagatgtctgagatgtcagaaacccttgaatcccgccgagaagctgagacacctgaacgagaagagaagattccacaagatcgccggccactacagagggcagtgccacagctgctgcaacagagctagacaagagagactgcagagaagacgggagacccaagtggctagaagggctgagcctcaaagacataccatgctgtgtatgtgctgcaaatgcgaggctagaatcgagctggtggtggagagcagcgccgacgacctgagagcctttcagcagctgttcctgagcaccctgagcttcgtgtgtccctggtgcgctagccaacagtgatga

SEQ ID NO: 54 - RNA, 3219 nt, synthetic construct
  source 1..3219: mol_type = other RNA
atggacgccatgaagcgcggtctttgctgcgtcctgctgttatgcggcgctgtgttcgtcagccctagcataacgcaggactgcagcttccagcacagccctatatcttcggacttcgcggtcaagattcgggagctctccgactatctgctccaggactatcccgtcacggtcgccagcaaccttcaggacgaagagttgtgtggcggcctgtggcggttagtcctggcgcagcgttggatggagcgcctgaagaccgtggctggttcgaagatgcagggcttgctggagcgggtgaacacggagattcacttcgtgaccaagtgcgcgtttcagcctccgccgagctgtctgaggttcgtgcagacgaacatcagtcggctcttgcaggagactagcgagcagttggtcgcgttgaagccgtggatcacccgccagaacttctcacgttgccttgagctgcagtgccagccggattcctcgaccctccctccgccgtggtcgccgcggccgctggaggccacggcgcccacggcgcctggcggcgggagcggagatatgaacgtgtgccaggataagatcttggagcattacgagaatgactccaaggatatcctggagcactatgagaacgactccaaggatctatgtgatcacatctgtgatcacatagattattggaagcacatccggctggagtgcgccattatgtataaggctcggatacggctggaatgtgctataatgtataaagcccgtgagatgggctttcaccagttcgatggtgacatttgtaacacaatgcactatacgaactggatatacatctgcgaggacgcgcagtgtacggtagttgagggtcaggtagacaagaagtgggaggttcacgcgggtgggcaggtcatcctctgcccggagtccgggcagaggaggatcaagcgtccgcggagtgaaaactgccaccctaacaagctactgatcctcaagtgccttcgctatcgcttcaagaagcattgcaagttgtcgtccacgtggcactggacttgccacgacggcaagcacaagtggcactggacgtgccacgacggcaagcacaagaacgcgatagtgacgcttacctatgatcacatagattattggaaagcgatccggcaggagaatgcgatattcttcgctgctagacaccaggtggtgcccgcgttgaatatctgcaaggcgaaggcctgcaaggccatagagtggaacacagagccgaagcactgctttaagaaaggcggtcagcacatcgaggtctggttcgactatgtggcctgggactcggtctactattgcggcgacgacggttggtgcaagaccgaggccgagaaatacggctgcaaagggacgtgggaagttcacttcgggaactccatcgattgcaacgactccatgtgcagcacgtttgacgataacgtgtctgccacggagttggtaaagatggcccgattcgaagatcccacaagaagaccctacaagctgcccgacctgtgcaccgagctgaacacaagcctccaagacatcgagattacctgcgtgtactgcaagaccgtgctggagctgaccgaggtgttcgagttcgccttcaaggacctgttcgtggtgtacagagacagcatcccacacgccgcctgccacaagtgcatcgacttctacagccggattcgggaactgcggtactacagcgacagcgtgatgtatgggcccaaggccaccctgcaagacatcgtgctgcacctggagcctcagaacgaaatacccgtggacctgctgtgccatgagcaactgagcgacagcgaggaagagaatgatgagatcgacggcgtgaatcatcagcacctgcccgctagaagggccgagccacaacggcacaccatgctgtgcatgtgcttctacagcagaatcagagaactccggtattacagcgactccgtgtacggagataccctcgagaagctgaccaacaccggcctgtacaatctgctgatcagatgtctgagatgtcagaaacccttaaatcccgccgagaagctgagacacctgaacgagaagagaagattccacaagatcgccggccactacagagggcagtgccacagctgctgcaacagagctagacaagagagactgcagagaagacgggagacccaagtggctagaagggctgagccgcaaagacataccatgctgtgtatgtgctgcaaatgcgaggctagaatcgagctggtggtggagagcagcgccgacgacctgagagcctttcagcagctgttcctgagcaccctgagcttcgtgtgtccctggtgcgctagccaacagatgcatcagaagagaaccgccatgttccaagatccgcaagagagacctagaaaactccctcatctgtgcaccgaactgcagaccaccatccacgacatcatcctggagtgcgtgtattgcaaacaacagctgctgagaagagaggtgtacgacttcgccttcagagacctgtgcatcgtgtaccgggacggcaatccctacgccgtgtgcgacaagtgcctcaagttctatagcaagatcagcgagtatagatacatgcacggagatacgccgaccctgcacgagtacatgctggacctgcagcccgagaccaccgacctgtactgctacgagcagctgaacgacagcagcgaagaggaggacgagattgacggcccggccggccaagccgagcccgacagagcccactacaacatcgtgaccttctgctgtaaatgcgatagcacactggacaagtgcctgaagttctacagcaagattagcgagtacagatattactgctactccgtgtacgggacaaccctggagcagcagtacaacaagcctctgtgcgacctgctgatccggtgtattaactgtcagaagcccttgtgtcccgaggagaagcagagacacctggacaagaagcagagattccacaacatcagaggcagatggaccggcagatgcatgagctgctgcagaagcagcagaacaagaagagagacacaactgcactacaatatcgtcaccttctgctgcaagtgcgactccacactgcggctctgcgtgcagagcacccacgtggacatcagaaccctggaggacctgctgatgggcaccctgggcatcgtgtgtcccatctgcagccaaaagccctgatga